European Patent Specification EP 3 853 241 B1, published October 4, 2023. Title: Site-specific serine ADP-ribosylated proteins and peptides and method for producing the same. Applicant: Max-Planck-Gesellschaft zur Förderung der Wissenschaften e.V. The sequence listing filed with the application follows.

SEQUENCE LISTING (309 sequences)

SEQ ID NO: 1 - protein, 1014 aa, Homo sapiens
  Poly (ADP-ribose) polymerase 1
MAESSDKLYRVEYAKSGRASCKKCSESIPKDSLRMAIMVQSPMFDGKVPHWYHFSCFWKVGHSIRHPDVEVDGFSELRWDDQQKVKKTAEAGGVTGKGQDGIGSKAEKTLGDFAAEYAKSNRSTCKGCMEKIEKGQVRLSKKMVDPEKPQLGMIDRWYHPGCFVKNREELGFRPEYSASQLKGFSLLATEDKEALKKQLPGVKSEGKRKGDEVDGVDEVAKKKSKKEKDKDSKLEKALKAQNDLIWNIKDELKKVCSTNDLKELLIFNKQQVPSGESAILDRVADGMVFGALLPCEECSGQLVFKSDAYYCTGDVTAWTKCMVKTQTPNRKEWVTPKEFREISYLKKLKVKKQDRIFPPETSASVAATPPPSTASAPAAVNSSASADKPLSNMKILTLGKLSRNKDEVKAMIEKLGGKLTGTANKASLCISTKKEVEKMNKKMEEVKEANIRVVSEDFLQDVSASTKSLQELFLAHILSPWGAEVKAEPVEVVAPRGKSGAALSKKSKGQVKEEGINKSEKRMKLTLKGGAAVDPDSGLEHSAHVLEKGGKVFSATLGLVDIVKGTNSYYKLQLLEDDKENRYWIFRSWGRVGTVIGSNKLEQMPSKEDAIEHFMKLYEEKTGNAWHSKNFTKYPKKFYPLEIDYGQDEEAVKKLTVNPGTKSKLPKPVQDLIKMIFDVESMKKAMVEYEIDLQKMPLGKLSKRQIQAAYSILSEVQQAVSQGSSDSQILDLSNRFYTLIPHDFGMKKPPLLNNADSVQAKVEMLDNLLDIEVAYSLLRGGSDDSSKDPIDVNYEKLKTDIKVVDRDSEEAEIIRKYVKNTHATTHNAYDLEVIDIFKIEREGECQRYKPFKQLHNRRLLWHGSRTTNFAGILSQGLRIAPPEAPVTGYMFGKGIYFADMVSKSANYCHTSQGDPIGLILLGEVALGNMYELKHASHISKLPKGKHSVKGLGKTTPDPSANISLDGVDVPLGTGISSGVNDTSLLYNEYIVYDIAQVNLKYLLKLKFNFKTSLW

SEQ ID NO: 2 - protein, 1014 aa, Artificial Sequence
  Poly (ADP-ribose) polymerase 1 E988Q
MAESSDKLYRVEYAKSGRASCKKCSESIPKDSLRMAIMVQSPMFDGKVPHWYHFSCFWKVGHSIRHPDVEVDGFSELRWDDQQKVKKTAEAGGVTGKGQDGIGSKAEKTLGDFAAEYAKSNRSTCKGCMEKIEKGQVRLSKKMVDPEKPQLGMIDRWYHPGCFVKNREELGFRPEYSASQLKGFSLLATEDKEALKKQLPGVKSEGKRKGDEVDGVDEVAKKKSKKEKDKDSKLEKALKAQNDLIWNIKDELKKVCSTNDLKELLIFNKQQVPSGESAILDRVADGMVFGALLPCEECSGQLVFKSDAYYCTGDVTAWTKCMVKTQTPNRKEWVTPKEFREISYLKKLKVKKQDRIFPPETSASVAATPPPSTASAPAAVNSSASADKPLSNMKILTLGKLSRNKDEVKAMIEKLGGKLTGTANKASLCISTKKEVEKMNKKMEEVKEANIRVVSEDFLQDVSASTKSLQELFLAHILSPWGAEVKAEPVEVVAPRGKSGAALSKKSKGQVKEEGINKSEKRMKLTLKGGAAVDPDSGLEHSAHVLEKGGKVFSATLGLVDIVKGTNSYYKLQLLEDDKENRYWIFRSWGRVGTVIGSNKLEQMPSKEDAIEHFMKLYEEKTGNAWHSKNFTKYPKKFYPLEIDYGQDEEAVKKLTVNPGTKSKLPKPVQDLIKMIFDVESMKKAMVEYEIDLQKMPLGKLSKRQIQAAYSILSEVQQAVSQGSSDSQILDLSNRFYTLIPHDFGMKKPPLLNNADSVQAKVEMLDNLLDIEVAYSLLRGGSDDSSKDPIDVNYEKLKTDIKVVDRDSEEAEIIRKYVKNTHATTHNAYDLEVIDIFKIEREGECQRYKPFKQLHNRRLLWHGSRTTNFAGILSQGLRIAPPEAPVTGYMFGKGIYFADMVSKSANYCHTSQGDPIGLILLGEVALGNMYELKHASHISKLPKGKHSVKGLGKTTPDPSANISLDGVDVPLGTGISSGVNDTSLLYNQYIVYDIAQVNLKYLLKLKFNFKTSLW

SEQ ID NO: 3 - protein, 1013 aa, Mus musculus
  Poly (ADP-ribose) polymerase 1, isoform 1
MAEASERLYRVQYAKSGRASCKKCSESIPKDSLRMAIMVQSPMFDGKVPHWYHFSCFWKVGQSIRHPDVEVDGFSELRWDDQQKVKKTAEAGGVAGKGQDGSGGKAEKTLGDFAAEYAKSNRSMCKGCLEKIEKGQMRLSKKMVDPEKPQLGMIDRWYHPTCFVKKRDELGFRPEYSASQLKGFSLLSAEDKEALKKQLPAIKNEGKRKGDEVDGTDEVAKKKSRKETDKYSKLEKALKAQNELIWNIKDELKKACSTNDLKELLIFNQQQVPSGESAILDRVADGMAFGALLPCKECSGQLVFKSDAYYCTGDVTAWTKCMVKTQNPSRKEWVTPKEFREISYLKKLKVKKQDRIFPPESSAPITVHWPLSVTSAPTAVNSSAPADKPLSNMKILTLGKLSQNKDEAKAVIEKLGGKLTGSANKASLCISIKKEVEKMNKKMEEVKEANIRVVSEDFLQDVSASTKSLQDLLSAHSLSPWGAEVKAEPGEVVAPRGKSAAPSKKSKGCFKEEGVNKSEKRMKLTLKGGAAVDPDSGLEHSAHVLEKGGKVFSATLGLVDIVKGTNSYYKLQLLEDDKESRYWIFRSWGRLGTVIGSNKLEQMPSKEEAVEQFMKLYEEKTGNAWHSKNFTKYPKKFYPLEIDYGQDEEAVKKLTVKPGTKSKLPKPVQELVGMIFDVDSMKKALVEYEIDLQKMPLGKLSRRQIQAAYSILSEVQQPVSQGSSESQILDLSNRFYTLIPHDFGMKKPPLLNNADSVQAKVEMLDNLLDIEVAYSLLRGGSDDSSKDPIDVNYEKLKTDIKVVDRDSEEAEVIRKYVKNTHATTHNAYDLEVIDIFKIEREGESQRYKPFRQLHNRRLLWHGSRTTNFAGILSQGLRIAPPEAPVTGYMFGKGIYFADMVSKSANYCHTSQGDPIGLIMLGEVALGNMYELKHASHISKLPKGKHSVKGLGKTTPDPSASITLEGVEVPLGTGIPSGVNDTALLYNEYIVYDIAQVNLKYLLKLKFNFKTSLW

SEQ ID NO: 4 - protein, 492 aa, Mus musculus
  Poly (ADP-ribose) polymerase 1, isoform 2
MKLTLKGGAAVDPDSGLEHSAHVLEKGGKVFSATLGLVDIVKGTNSYYKLQLLEDDKESRYWIFRSWGRLGTVIGSNKLEQMPSKEEAVEQFMKLYEEKTGNAWHSKNFTKYPKKFYPLEIDYGQDEEAVKKLTVKPGTKSKLPKPVQELVGMIFDVDSMKKALVEYEIDLQKMPLGKLSRRQIQAAYSILSEVQQPVSQGSSESQILDLSNRFYTLIPHDFGMKKPPLLNNADSVQAKVEMLDNLLDIEVAYSLLRGGSDDSSKDPIDVNYEKLKTDIKVVDRDSEEAEVIRKYVKNTHATTHNAYDLEVIDIFKIEREGESQRYKPFRQLHNRRLLWHGSRTTNFAGILSQGLRIAPPEAPVTGYMFGKGIYFADMVSKSANYCHTSQGDPIGLIMLGEVALGNMYELKHASHISKLPKGKHSVKGLGKTTPDPSASITLEGVEVPLGTGIPSGVNDTALLYNEYIVYDIAQVNLKYLLKLKFNFKTSLW

SEQ ID NO: 5 - protein, 1014 aa, Rattus norvegicus
  Poly (ADP-ribose) polymerase 1
MAEATERLYRVEYAKSGRASCKKCSESIPKDSLRMAIMVQSPMFDGKVPHWYHFSCFWKVGHSIRQPDTEVDGFSELRWDDQQKVKKTAEAGGVAGKGQHGGGGKAEKTLGDFAAEYAKSNRSTCKGCMEKIEKGQMRLSKKMLDPEKPQLGMIDRWYHPTCFVKNRDELGFRPEYSASQLKGFSLLSAEDKEALKKQLPAVKSEGKRKCDEVDGIDEVAKKKSKKGKDKESSKLEKALKAQNELVWNIKDELKKACSTNDLKELLIFNQQQVPSGESAILDRVADGMAFGALLPCKECSGQLVFKSDAYYCTGDVTAWTKCMVKTQNPSRKEWVTPKEFREISYLKKLKIKKQDRLFPPESSAPAPPAPPVSITSAPTAVNSSAPADKPLSNMKILTLGKLSQNKDEAKAMIEKLGGKLTGSANKASLCISTKKEVEKMSKKMEEVKAANVRVVCEDFLQDVSASAKSLQELLSAHSLSSWGAEVKVEPGEVVVPKGKSAAPSKKSKGAVKEEGVNKSEKRMKLTLKGGAAVDPDSGLEHSAHVLEKGGKVFSATLGLVDIVKGTNSYYKLQLLESDKESRYWIFRSWGRVGTVIGSNKLEQMPSKEDAVEHFMKLYEEKTGNAWHSKNFTKYPKKFYPLEIDYGQDEEAVKKLAVKPGTKSKLPKPVQELVGMIFDVESMKKALVEYEIDLQKMPLGKLSRRQIQAAYSILSEVQQAVSQGSSESQILDLSNRFYTLIPHDFGMKKPPLLNNTDSVQAKVEMLDNLLDIEVAYSLLRGGSDDSSKDPIDVNYEKLKTDIKVVDRDSEEAEVIRKYVKNTHATTHNAYDLEVIDIFKIEREGESQRYKPFRQLHNRRLLWHGSRTTNFAGILSQGLRIAPPEAPVTGYMFGKGIYFADMVSKSANYCHTSQGDPIGLILLGEVALGNMYELKHASHISKLPKGKHSVKGLGKTAPDPSASITLDGVEVPLGTGIPSGVNDTCLLYNEYIVYDIAQVNLKYLLKLKFNFKTSLW

SEQ ID NO: 6 - protein, 583 aa, Homo sapiens
  Poly (ADP-ribose) polymerase 2, isoform 1
MAARRRRSTGGGRARALNESKRVNNGNTAPEDSSPAKKTRRCQRQESKKMPVAGGKANKDRTEDKQDGMPGRSWASKRVSESVKALLLKGKAPVDPECTAKVGKAHVYCEGNDVYDVMLNQTNLQFNNNKYYLIQLLEDDAQRNFSVWMRWGRVGKMGQHSLVACSGNLNKAKEIFQKKFLDKTKNNWEDREKFEKVPGKYDMLQMDYATNTQDEEETKKEESLKSPLKPESQLDLRVQELIKLICNVQAMEEMMMEMKYNTKKAPLGKLTVAQIKAGYQSLKKIEDCIRAGQHGRALMEACNEFYTRIPHDFGLRTPPLIRTQKELSEKIQLLEALGDIEIAIKLVKTELQSPEHPLDQHYRNLHCALRPLDHESYEFKVISQYLQSTHAPTHSDYTMTLLDLFEVEKDGEKEAFREDLHNRMLLWHGSRMSNWVGILSHGLRIAPPEAPITGYMFGKGIYFADMSSKSANYCFASRLKNTGLLLLSEVALGQCNELLEANPKAEGLLQGKHSTKGLGKMAPSSAHFVTLNGSTVPLGPASDTGILNPDGYTLNYNEYIVYNPNQVRMRYLLKVQFNFLQLW

SEQ ID NO: 7 - protein, 570 aa, Homo sapiens
  Poly (ADP-ribose) polymerase 2, isoform 2
MAARRRRSTGGGRARALNESKRVNNGNTAPEDSSPAKKTRRCQRQESKKMPVAGGKANKDRTEDKQDESVKALLLKGKAPVDPECTAKVGKAHVYCEGNDVYDVMLNQTNLQFNNNKYYLIQLLEDDAQRNFSVWMRWGRVGKMGQHSLVACSGNLNKAKEIFQKKFLDKTKNNWEDREKFEKVPGKYDMLQMDYATNTQDEEETKKEESLKSPLKPESQLDLRVQELIKLICNVQAMEEMMMEMKYNTKKAPLGKLTVAQIKAGYQSLKKIEDCIRAGQHGRALMEACNEFYTRIPHDFGLRTPPLIRTQKELSEKIQLLEALGDIEIAIKLVKTELQSPEHPLDQHYRNLHCALRPLDHESYEFKVISQYLQSTHAPTHSDYTMTLLDLFEVEKDGEKEAFREDLHNRMLLWHGSRMSNWVGILSHGLRIAPPEAPITGYMFGKGIYFADMSSKSANYCFASRLKNTGLLLLSEVALGQCNELLEANPKAEGLLQGKHSTKGLGKMAPSSAHFVTLNGSTVPLGPASDTGILNPDGYTLNYNEYIVYNPNQVRMRYLLKVQFNFLQLW

SEQ ID NO: 8 - protein, 559 aa, Mus musculus
  Poly (ADP-ribose) polymerase 2
MAPRRQRSGSGRRVLNEAKKVDNGNKATEDDSPPGKKMRTCQRKGPMAGGKDADRTKDNRDSVKTLLLKGKAPVDPECAAKLGKAHVYCEGDDVYDVMLNQTNLQFNNNKYYLIQLLEDDAQRNFSVWMRWGRVGKTGQHSLVTCSGDLNKAKEIFQKKFLDKTKNNWEDRENFEKVPGKYDMLQMDYAASTQDESKTKEEETLKPESQLDLRVQELLKLICNVQTMEEMMIEMKYDTKRAPLGKLTVAQIKAGYQSLKKIEDCIRAGQHGRALVEACNEFYTRIPHDFGLSIPPVIRTEKELSDKVKLLEALGDIEIALKLVKSERQGLEHPLDQHYRNLHCALRPLDHESNEFKVISQYLQSTHAPTHKDYTMTLLDVFEVEKEGEKEAFREDLPNRMLLWHGSRLSNWVGILSHGLRVAPPEAPITGYMFGKGIYFADMSSKSANYCFASRLKNTGLLLLSEVALGQCNELLEANPKAQGLLRGKHSTKGMGKMAPSPAHFITLNGSTVPLGPASDTGILNPEGYTLNYNEFIVYSPNQVRMRYLLKIQFNFLQLW

SEQ ID NO: 9 - protein, 346 aa, Homo sapiens [sequence omitted]

SEQ ID NO: 10 - protein, 346 aa, Mus musculus
  Histone PARylation factor 1
MVGGGGKRRTAGAGPQCEKTVEVKKSKFSEADVSSDLRKEVENLYKLSLPEDFYHFWKFCEELDPEKPADALATSLGLRLVGPYDILAGKHKMKKKPTGLNCNLHWRFYYDPPEFQTIIIGDNKTQYHMGYFRDSPDELPVYVGTNEAKKNCIIIQNGDNVFAAIKLFLMKKLKEVTDRKKISILKNIDEKLTEAARKLGYSLEQRTVKMRQRDKKVVTKTFHGAGLVVPVDKNDVGYRELPETDADLKRICKAVVDAASDEERLKAFAPIQEMMTFVQFANDECDYGMGLELGMDLFCYGSHYFHKVAGQLLPLAYNLLKRDLFAKIIEDHLASRSEENIDQLAG

SEQ ID NO: 11 - protein, 976 aa, Homo sapiens
  Poly (ADP-ribose) glycohydrolase, isoform 1
MNAGPGCEPCTKRPRWGAATTSPAASDARSFPSRQRRVLDPKDAHVQFRVPPSSPACVPGRAGQHRGSATSLVFKQKTITSWMDTKGIKTAESESLDSKENNNTRIESMMSSVQKDNFYQHNVEKLENVSQLSLDKSPTEKSTQYLNQHQTAAMCKWQNEGKHTEQLLESEPQTVTLVPEQFSNANIDRSPQNDDHSDTDSEENRDNQQFLTTVKLANAKQTTEDEQAREAKSHQKCSKSCDPGEDCASCQQDEIDVVPESPLSDVGSEDVGTGPKNDNKLTRQESCLGNSPPFEKESEPESPMDVDNSKNSCQDSEADEETSPGFDEQEDGSSSQTANKPSRFQARDADIEFRKRYSTKGGEVRLHFQFEGGESRTGMNDLNAKLPGNISSLNVECRNSKQHGKKDSKITDHFMRLPKAEDRRKEQWETKHQRTERKIPKYVPPHLSPDKKWLGTPIEEMRRMPRCGIRLPLLRPSANHTVTIRVDLLRAGEVPKPFPTHYKDLWDNKHVKMPCSEQNLYPVEDENGERTAGSRWELIQTALLNKFTRPQNLKDAILKYNVAYSKKWDFTALIDFWDKVLEEAEAQHLYQSILPDMVKIALCLPNICTQPIPLLKQKMNHSITMSQEQIASLLANAFFCTFPRRNAKMKSEYSSYPDINFNRLFEGRSSRKPEKLKTLFCYFRRVTEKKPTGLVTFTRQSLEDFPEWERCEKPLTRLHVTYEGTIEENGQGMLQVDFANRFVGGGVTSAGLVQEEIRFLINPELIISRLFTEVLDHNECLIITGTEQYSEYTGYAETYRWSRSHEDGSERDDWQRRCTEIVAIDALHFRRYLDQFVPEKMRRELNKAYCGFLRPGVSSENLSAVATGNWGCGAFGGDARLKALIQILAAAAAERDVVYFTFGDSELMRDIYSMHIFLTERKLTVGDVYKLLLRYYNEECRNCSTPGPDIKLYPFIYHAVESCAETADHSGQRTGT

SEQ ID NO: 12 - protein, 894 aa, Homo sapiens
  Poly (ADP-ribose) polymerase 1, isoform 2
MDTKGIKTAESESLDSKENNNTRIESMMSSVQKDNFYQHNVEKLENVSQLSLDKSPTEKSTQYLNQHQTAAMCKWQNEGKHTEQLLESEPQTVTLVPEQFSNANIDRSPQNDDHSDTDSEENRDNQQFLTTVKLANAKQTTEDEQAREAKSHQKCSKSCDPGEDCASCQQDEIDVVPESPLSDVGSEDVGTGPKNDNKLTRQESCLGNSPPFEKESEPESPMDVDNSKNSCQDSEADEETSPGFDEQEDGSSSQTANKPSRFQARDADIEFRKRYSTKGGEVRLHFQFEGGESRTGMNDLNAKLPGNISSLNVECRNSKQHGKKDSKITDHFMRLPKAEDRRKEQWETKHQRTERKIPKYVPPHLSPDKKWLGTPIEEMRRMPRCGIRLPLLRPSANHTVTIRVDLLRAGEVPKPFPTHYKDLWDNKHVKMPCSEQNLYPVEDENGERTAGSRWELIQTALLNKFTRPQNLKDAILKYNVAYSKKWDFTALIDFWDKVLEEAEAQHLYQSILPDMVKIALCLPNICTQPIPLLKQKMNHSITMSQEQIASLLANAFFCTFPRRNAKMKSEYSSYPDINFNRLFEGRSSRKPEKLKTLFCYFRRVTEKKPTGLVTFTRQSLEDFPEWERCEKPLTRLHVTYEGTIEENGQGMLQVDFANRFVGGGVTSAGLVQEEIRFLINPELIISRLFTEVLDHNECLIITGTEQYSEYTGYAETYRWSRSHEDGSERDDWQRRCTEIVAIDALHFRRYLDQFVPEKMRRELNKAYCGFLRPGVSSENLSAVATGNWGCGAFGGDARLKALIQILAAAAAERDVVYFTFGDSELMRDIYSMHIFLTERKLTVGDVYKLLLRYYNEECRNCSTPGPDIKLYPFIYHAVESCAETADHSGQRTGT

SEQ ID NO: 13 - protein, 868 aa, Homo sapiens
  Poly (ADP-ribose) glycohydrolase, isoform 3
MMSSVQKDNFYQHNVEKLENVSQLSLDKSPTEKSTQYLNQHQTAAMCKWQNEGKHTEQLLESEPQTVTLVPEQFSNANIDRSPQNDDHSDTDSEENRDNQQFLTTVKLANAKQTTEDEQAREAKSHQKCSKSCDPGEDCASCQQDEIDVVPESPLSDVGSEDVGTGPKNDNKLTRQESCLGNSPPFEKESEPESPMDVDNSKNSCQDSEADEETSPGFDEQEDGSSSQTANKPSRFQARDADIEFRKRYSTKGGEVRLHFQFEGGESRTGMNDLNAKLPGNISSLNVECRNSKQHGKKDSKITDHFMRLPKAEDRRKEQWETKHQRTERKIPKYVPPHLSPDKKWLGTPIEEMRRMPRCGIRLPLLRPSANHTVTIRVDLLRAGEVPKPFPTHYKDLWDNKHVKMPCSEQNLYPVEDENGERTAGSRWELIQTALLNKFTRPQNLKDAILKYNVAYSKKWDFTALIDFWDKVLEEAEAQHLYQSILPDMVKIALCLPNICTQPIPLLKQKMNHSITMSQEQIASLLANAFFCTFPRRNAKMKSEYSSYPDINFNRLFEGRSSRKPEKLKTLFCYFRRVTEKKPTGLVTFTRQSLEDFPEWERCEKPLTRLHVTYEGTIEENGQGMLQVDFANRFVGGGVTSAGLVQEEIRFLINPELIISRLFTEVLDHNECLIITGTEQYSEYTGYAETYRWSRSHEDGSERDDWQRRCTEIVAIDALHFRRYLDQFVPEKMRRELNKAYCGFLRPGVSSENLSAVATGNWGCGAFGGDARLKALIQILAAAAAERDVVYFTFGDSELMRDIYSMHIFLTERKLTVGDVYKLLLRYYNEECRNCSTPGPDIKLYPFIYHAVESCAETADHSGQRTGT

SEQ ID NO: 14 - protein, 969 aa, Mus musculus
  Poly (ADP-ribose) glycohydrolase, isoform 1
MSAGPGWEPCTKRPRWGAAGTSAPTASDSRSFPGRQRRVLDPKDAPVQFRVPPSSPACVSGRAGPHRGNATSFVFKQKTITTWMDTKGPKTAESESKENNNTRIDSMMSSVQKDNFYPHKVEKLENVPQLNLDKSPTEKSSQYLNQQQTASVCKWQNEGKHAEQLLASEPPAGTPLPKQLSNANIGQSPHTDDHSDTDHEEDRDNQQFLTPIKLANTKPTVGDGQARSNCKCSGSRQSVKDCTGCQQEEVDVLPESPLSDVGAEDIGTGPKNDNKLTGQESSLGDSPPFEKESEPESPMDVDNSKNSCQDSEADEETSPVFDEQDDRSSQTANKLSSCQAREADGDLRKRYLTKGSEVRLHFQFEGENNAGTSDLNAKPSGNSSSLNVECRSSKQHGKRDSKITDHFMRISKSEDRRKEQCEVRHQRTERKIPKYIPPNLPPEKKWLGTPIEEMRKMPRCGIHLPSLRPSASHTVTVRVDLLRAGEVPKPFPTHYKDLWDNKHVKMPCSEQNLYPVEDENGERTAGSRWELIQTALLNKFTRPQNLKDAILKYNVAYSKKWDFTALVDFWDKVLEEAEAQHLYQSILPDMVKIALCLPNICTQPIPLLKQKMNHSVTMSQEQIASLLANAFFCTFPRRNAKMKSEYSSYPDINFNRLFEGRSSRKPEKLKTLFCYFRRVTEKKPTGLVTFTRQSLEDFPEWERCEKPLTRLHVTYEGTIEGNGRGMLQVDFANRFVGGGVTGAGLVQEEIRFLINPELIVSRLFTEVLDHNECLIITGTEQYSEYTGYAETYRWARSHEDGSEKDDWQRRCTEIVAIDALHFRRYLDQFVPEKVRRELNKAYCGFLRPGVPSENLSAVATGNWGCGAFGGDARLKALIQILAAAAAERDVVYFTFGDSELMRDIYSMHTFLTERKLDVGKVYKLLLRYYNEECRNCSTPGPDIKLYPFIYHAVESSAETTDMPGQKAGT

SEQ ID NO: 15 - protein, 920 aa, Mus musculus
  Poly (ADP-ribose) glycohydrolase, isoform 2
MSAGPGWEPCTKRPRWGAAGTSAPTASDSRSFPGRQRRVLDPKDAPVQFRVPPSSPACVSGRAGPHRGNATSFVFKQKTITTWMDTKGPKTAESESKENNNTRIDSMMSSVQKDNFYPHKVEKLENVPQLNLDKSPTEKSSQYLNQQQTASVCKWQNEGKHAEQLLASEPPAGTPLPKQLSNANIGQSPHTDDHSDTDHEEDRDNQQFLTPIKLANTKPTVGDGQARSNCKCSGSRQSVKDCTGCQQEEVDVLPESPLSDVGAEDIGTGPKNDNKLTGQESSLGDSPPFEKESEPESPMDVDNSKNSCQDSEADEETSPVFDEQDDRSSQTANKLSSCQAREADGDLRKRYLTKGSEVRLHFQFEGENNAGTSDLNAKPSGNSSSLNVECRSSKQHGKRDSKITDHFMRISKSEDRRKEQCEVRHQRTERKIPKYIPPNLPPEKKWLGTPIEEMRKMPRCGIHLPSLRPSASHTVTVRVDLLRAGEVPKPFPTHYKDLWDNKHVKMPCSEQNLYPVEDENGERTAGSRWELIQTALLNKFTRPQNLKDAILKYNVAYSKKWDFTALVDFWDKVLEEAEAQHLYQSILPDMVKIALCLPNICTQPIPLLKQKMNHSVTMSQEQIASLLANAFFCTFPRRNAKMKSEYSSYPDINFNRLFEGRSSRKPEKLKTLFCYFRRVTEKKPTGLVTFTRQSLEDFPEWERCEKPLTRLHVTYEGTIEGNGRGMLQVDFANRFVGGGVTGAGLVQEEIRFLINPELIVSRLFTEVLDHNECLIITGTEQYSEYTGYAETYRWARSHEDGSEKDDWQRRCTEIVAIDALHFRRYLDQFVPEKVRRELNKAYCGFLRPGVPSENLSAVATGNWGCGAFGGDARLKALIQILAAAAAERDVVYFTFGDSELMRDIYSMHTFLTERKLDVGE

SEQ ID NO: 16 - protein, 972 aa, Rattus norvegicus
  Poly (ADP-ribose) glycohydrolase
MSAGPGCEPCTKRPRWGAAGTSAPTASDSRSFPGRQKRVLDPKDAPVQFRVPPSSSACVSGRAGPHRGSVTSFVFKQKPITTWMDTKGPKTAESESKENNNTRTDPMMSSVQKDNFYPHKVEKLGNVPQLNLDKSPTEKSTPYLNQQQTAGVCKWHSAGERAEQLSASEPSAVTQAPKQLSNANIDQSPPTDGHSDTDHEEDRDNQQFLTPVKLANAKQTVGDGQARSNCKCSASCQCGQDCAGCQREEADVIPESPLSDVGAEDIGTGSKNDNKLTGQESGLGDSPPFEKESEPESPMDVDNSKTSCQDSEADEEASPVFDEQDDQDDRSSQTANKLSSRQAREVDGDLRKRYLTKGSEIRLHFQFEGGSNAGTSDLNAKPSGNSSSLNVDGRSSKQHGKRDSKITDHFVRIPKSEDKRKEQCEVRHQRAERKIPKYVPPNLPPDKKWLGTPIEEMRKMPRCGVRLPLLRPSASHTVTVRVDLLRAGEVPKPFPTHYKDLWDNKHVKMPCSEQNLYPVEDENGERTAGSRWELIQTALLNKFTRPQNLKDAILKYNVAYSKKWDFTALVDFWDKVLEEAEAQHLYQSILPDMVKIALCLPNICTQPIPLLKQKMNHSVTMSQEQIASLLANAFFCTFPRRNAKMKSEYSSYPDINFNRLFEGRSSRKPEKLKTLFCYFRRVTEKKPTGLVTFTRQSLEDFPEWERCDKPLTRLHVTYEGTIEGNGRGMLQVDFANRFVGGGVTGAGLVQEEIRFLINPELIVSRLFTEVLDHNECLIITGTEQYSEYTGYAETYRWARSHEDGSEKDDWQRCCTEIVAIDALHFRRYLDQFVPEKVRRELNKAYCGFLRPGVPPENLSAVATGNWGCGAFGGDARLKALIQLLAAAAAERDVVYFTFGDSELMRDIYSMHTFLTERKLNVGKVYRLLLRYYREECRDCSSPGPDTKLYPFIYHAAESSAETSDQPGQRTGT

SEQ ID NO: 17 - protein, 16 aa, Homo sapiens
  Poly [ADP-ribose] polymerase 1
APRGKSGAALSKKSKG

SEQ ID NO: 18 - protein, 18 aa, Homo sapiens
  Poly [ADP-ribose] polymerase 1
KKSKGQVKEEGINKSEKR

SEQ ID NO: 19 - protein, 23 aa, Homo sapiens
  Poly [ADP-ribose] polymerase 1
GSKAEKTLGDFAAEYAKSNRSTC

SEQ ID NO: 20 - protein, 34 aa, Homo sapiens
  Poly [ADP-ribose] polymerase 1
GVKSEGKRKGDEVDGVDEVAKKKSKKEKDKDSKL

SEQ ID NO: 21 - protein, 25 aa, Homo sapiens
  Histone H3.1
ARKSTGGKAPRKQLATKAARKSAPA

SEQ ID NO: 22 - protein, 25 aa, Homo sapiens
  Histone H3.2
ARKSTGGKAPRKQLATKAARKSAPA

SEQ ID NO: 23 - protein, 25 aa, Homo sapiens
  Histone H3.3
ARKSTGGKAPRKQLATKAARKSAPS

SEQ ID NO: 24 - protein, 25 aa, Homo sapiens
  Histone H3.3C
ARKSTGGKAPRKQLATKAARKSTPS

SEQ ID NO: 25 - protein, 25 aa, Homo sapiens
  Histone H3.1t
ARKSTGGKAPRKQLATKVARKSAPA

SEQ ID NO: 26 - protein, 19 aa, Homo sapiens
  Histone H2B type 1-C/E/F/G/I
PEPAKSAPAPKKGSKKAVT

SEQ ID NO: 27 - protein, 49 aa, Homo sapiens
  Histone H4
SGRGKGGKGLGKGGAKRHRKVLRDNIQGITKPAIRRLARRGGVKRISGL

SEQ ID NO: 28 - protein, 21 aa, Homo sapiens
  Histone H2A type 1-B/E
SGRGKQGGKARAKAKTRSSRA

SEQ ID NO: 29 - protein, 21 aa, Homo sapiens
  Histone H2A type 1
SGRGKQGGKARAKAKTRSSRA

SEQ ID NO: 30 - protein, 21 aa, Homo sapiens
  Histone H2A type 1-D
SGRGKQGGKARAKAKTRSSRA

SEQ ID NO: 31 - protein, 33 aa, Homo sapiens
  Histone H1.0
KKSVAFKKTKKEIKKVATPKKASKPKKAASKAP

SEQ ID NO: 32 - protein, 19 aa, Homo sapiens
  Histone H1.2 (consensus with other histones)
KSPKKAKVAKPKKAAKSAA

SEQ ID NO: 33 - protein, 25 aa, Homo sapiens
  Histone H1.4
KKSAKKTPKKAKKPAAAAGAKKAKS

SEQ ID NO: 34 - protein, 6 aa, Homo sapiens
  Histone H1.4 (consensus with other histones)
ERSGVS

SEQ ID NO: 35 - protein, 11 aa, Homo sapiens
  Histone H1.4 (consensus with other histones)
SFKLNKKAASG

SEQ ID NO: 36 - protein, 27 aa, Homo sapiens
  Nucleophosmin
AQKSNQNGKDSKPSSTPRSKGQESFKK

SEQ ID NO: 37 - protein, 63 aa, Homo sapiens
  Translation machinery-associated protein 7
SGREGGKKKPLKQPKKQAKEMDEEDKAFKQKQKEEQKKLEELKAKAAGKGPLATGGIKKSGKK

SEQ ID NO: 38 - protein, 19 aa, Homo sapiens
  Protein DEK
TSKSKKSVKSANVKKADSS

SEQ ID NO: 39 - protein, 9 aa, Homo sapiens
  Heterogeneous nuclear ribonucleoprotein U
AAGKSSGPT

SEQ ID NO: 40 - protein, 23 aa, Homo sapiens
  Translation machinery-associated protein 16
PKAPKGKSAGREKKVIHPYSRKA

SEQ ID NO: 41 - protein, 12 aa, Homo sapiens
  HMGA1 (High mobility group protein HMG-I/HMG-Y)
SSSKSSQPLASK

SEQ ID NO: 42 - protein, 12 aa, Homo sapiens
  HMGA1 (High mobility group protein HMG-I/HMG-Y)
VSPGTALVGSQK

SEQ ID NO: 43 - protein, 9 aa, Homo sapiens
  HMGN1 (Non-histone chromosomal protein HMG-14)
KRKVSSAEG

SEQ ID NO: 44 - protein, 9 aa, Homo sapiens
  HMGN2 (Non-histone chromosomal protein HMG-17)
RRSARLSAK

SEQ ID NO: 45 - protein, 17 aa, Homo sapiens
  High mobility group protein B1
SEYRPKIKGEHPGLSIG

SEQ ID NO: 46 - protein, 17 aa, Homo sapiens
  Actin-related protein 8
SAKATADRKSASKPIGF

SEQ ID NO: 47 - protein, 26 aa, Homo sapiens
  Activity-dependent neuroprotector homeobox protein
SSVHLQQNNYGVKSVGQGYSVGQSMR

SEQ ID NO: 48 - protein, 31 aa, Homo sapiens
  Activity-dependent neuroprotector homeobox protein
KPQPKVQEKADIPVKSSPQAAVPYKKDVGKT

SEQ ID NO: 49 - protein, 31 aa, Homo sapiens
  Protein ELYS
QELQITTGRESKRLKSSQLLEPAVEETTKKE

SEQ ID NO: 50 - protein, 31 aa, Homo sapiens
  RNA demethylase ALKBH5
HRPRILEMDKEENRRSVLLPTHRRRGSFSSE

SEQ ID NO: 51 - protein, 31 aa, Homo sapiens
  RNA demethylase ALKBH5
ILRKTRLDAPRLETKSLSSSVLPPSYASDRL

SEQ ID NO: 52 - protein, 31 aa, Homo sapiens
  Ankyrin repeat domain-containing protein 11
DKNSEKRKEQTEKHKSVPGYLSEKDKKRRES

SEQ ID NO: 53 - protein, 31 aa, Homo sapiens
  DNA-(apurinic or apyrimidinic site) lyase 2
SEAKDEKELRTSFWKSVLAGPLRTPLCGGHR

SEQ ID NO: 54 - protein, 31 aa, Homo sapiens
  ATPase family AAA domain-containing protein 5
ESKARDKGNNPETKKSIPCPPKTTAGKKCSA

SEQ ID NO: 55 - protein, 27 aa, Homo sapiens
  Arginine vasopressin-induced protein 1
HSRKKSARIRRNWRKSGPTSYLHQIRH

SEQ ID NO: 56 - protein, 23 aa, Homo sapiens
  Bromo adjacent homology domain-containing 1 protein
MTHTRRKSLPMLSSGLTGRREPL

SEQ ID NO: 57 - protein, 31 aa, Homo sapiens
  BRCA1-associated RING domain protein 1
CCAARVDLKEDKPRKSLFNDAGNKKNSIKMW

SEQ ID NO: 58 - protein, 31 aa, Homo sapiens
  Bcl-2-associated transcription factor 1
DYRQFRKSVLADQGKSFATASHRNTEEEGLK

SEQ ID NO: 59 - protein, 31 aa, Homo sapiens
  Bcl-2-associated transcription factor 1
GDDTEETEDYRQFRKSVLADQGKSFATASHR

SEQ ID NO: 60 - protein, 31 aa, Homo sapiens
  BCL-6 corepressor-like protein 1
TQRDTQYRSHHAQDKSLLSQGRRHLWRAREM

SEQ ID NO: 61 - protein, 31 aa, Homo sapiens
  Bloom syndrome protein
KGGSATCRKISSKTKSSSIIGSSSASHTSQA

SEQ ID NO: 62 - protein, 31 aa, Homo sapiens
  Bloom syndrome protein
DWDDMDDFDTSETSKSFVTPPQSHFVRVSTA

SEQ ID NO: 63 - protein, 31 aa, Homo sapiens
  Bromodomain-containing protein 3
KELEKRLQDVSGQLSSSKKPARKEKPGSAPS

SEQ ID NO: 64 - protein, 31 aa, Homo sapiens
  Uncharacterized protein C1orf131
KKKRKGQEDRKSKKKSAPSILSNGRIGQVGK

SEQ ID NO: 65 - protein, 31 aa, Homo sapiens
  Uncharacterized protein C1orf131
EPSPLPGSLIRGQRKSASSFFKELREERHCA

SEQ ID NO: 66 - protein, 31 aa, Homo sapiens
  Caldesmon
DSRLEQYTSAIEGTKSAKPTKPAASDLPVPA

SEQ ID NO: 67 - protein, 31 aa, Homo sapiens
  Coiled-coil domain-containing protein 86
PKSGRVWKDRSKKRFSQMLQDKPLRTSWQRK

SEQ ID NO: 68 - protein, 31 aa, Homo sapiens
  DNA-directed RNA polymerase I subunit RPA34
RFCAFGGNPPVTGPRSALAPNLLTSGKKKKE

SEQ ID NO: 69 - protein, 31 aa, Homo sapiens
  Cell division cycle protein 20 homolog
NLNGFDVEEAKILRLSGKPQNAPEGYQNRLK

SEQ ID NO: 70 - protein, 31 aa, Homo sapiens
  Cell division cycle protein 27 homolog
PSKKSVARIGQTGTKSVFSQSGNSREVTPIL

SEQ ID NO: 71 - protein, 31 aa, Homo sapiens
  Cell division cycle-associated protein 2
ANTKATSQFKGYRRRSSLNGKGESSLTALER

SEQ ID NO: 72 - protein, 31 aa, Homo sapiens
  Cell division cycle-associated protein 2
GPAAGSSDEPGKRRKSFCISTLANTKATSQF

SEQ ID NO: 73 - protein, 31 aa, Homo sapiens
  Cell division cycle-associated protein 2
SCRKKKGKGKKSVQKSLYGERDIASKKPLLS

SEQ ID NO: 74 - protein, 31 aa, Homo sapiens
  Cyclin-dependent kinase 13
RSRHSSISPSTLTLKSSLAAELNKNKKARAA

SEQ ID NO: 75 - protein, 31 aa, Homo sapiens
  CDKN2A-interacting protein
FFVPLKELADLPQNKSSQESIVCELRCKSVY

SEQ ID NO: 76 - protein, 31 aa, Homo sapiens
  Centromere protein V
RSRSSAAAKLRGQKRSGASAAPAASAAAALA

SEQ ID NO: 77 - protein, 31 aa, Homo sapiens
  CGG triplet repeat-binding protein 1
LFCTSCNVVLNHVRKSAISDHLKSKTHTKRK

SEQ ID NO: 78 - protein, 31 aa, Homo sapiens
  Chromatin assembly factor 1 subunit A
VVLQDILAVRPPQIKSLPATPQGKNMTPESE

SEQ ID NO: 79 - protein, 31 aa, Homo sapiens
  Chromosome alignment-maintaining phosphoprotein 1
ESQKSSRGGSPDLWKSSFFIEPQKPVFPETR

SEQ ID NO: 80 - protein, 31 aa, Homo sapiens
  Chromosome alignment-maintaining phosphoprotein 1
PSSWKSPPASPESWKSGPPELRKTAPTLSPE

SEQ ID NO: 81 - protein, 31 aa, Homo sapiens
  Chromodomain-helicase-DNA-binding protein 1
VQAKPPKVDGAEFWKSSPSILAVQRSAILKK

SEQ ID NO: 82 - protein, 31 aa, Homo sapiens
  Chromodomain Helicase DNA Binding Protein 1 Like
ARGIPTYIYYFPRSKSAVLHSQSSSSSSRQL

SEQ ID NO: 83 - protein, 31 aa, Homo sapiens
  Chromodomain-helicase-DNA-binding protein 2
KDHHYGDRRHMDAHRSGSYRPNNMSRKRPYD

SEQ ID NO: 84 - protein, 31 aa, Homo sapiens
  Chromodomain-helicase-DNA-binding protein 7
TADGQTRALVNHSGLSAPVPRGRKGKKVKAQ

SEQ ID NO: 85 - protein, 31 aa, Homo sapiens
  Chromodomain-helicase-DNA-binding protein 7
ITPTADGQTRALVNHSGLSAPVPRGRKGKKV

SEQ ID NO: 86 - protein, 31 aa, Homo sapiens
  Chromodomain-helicase-DNA-binding protein 9
ELQSASETSLVNFPKSIPVSGTSIQPTLGAN

SEQ ID NO: 87 - protein, 31 aa, Homo sapiens
  Chromosome transmission fidelity protein 8 homolog isoform 2
LNPASFPRMNGPAGKSFVPFPRVGSLPGTNP

SEQ ID NO: 88 - protein, 31 aa, Homo sapiens
  Anamorsin
EVGSSRQLKLSITKKSSPSVKPAVDPAAAKL

SEQ ID NO: 89 - protein, 31 aa, Homo sapiens
  Cullin-4B
SPTAATSQQQQLKNKSILISSVASVHHANGL

SEQ ID NO: 90 - protein, 18 aa, Homo sapiens
  Cullin-4B
MKSVCPVTSGFSSPSPSA

SEQ ID NO: 91 - protein, 18 aa, Homo sapiens
  Pre-mRNA-splicing factor CWC22 homolog
MKSSVAQIKPSSGHDRRE

SEQ ID NO: 92 - protein, 31 aa, Homo sapiens
  CXXC-type zinc finger protein 1
GVGAMLARGSASPHKSSPQPLVATPSQHHQQ

SEQ ID NO: 93 - protein, 31 aa, Homo sapiens
  CXXC-type zinc finger protein 5
ASVADDTPPPERRNKSGIISEPLNKSLRRSR

SEQ ID NO: 94 - protein, 31 aa, Homo sapiens
  DDB1- and CUL4-associated factor 13
YPHIKRIARHRHLPKSIYSQIQEQRIMKEAR

SEQ ID NO: 95 - protein, 31 aa, Homo sapiens
  Probable ATP-dependent RNA helicase DDX27
EPVRGPAKKQKQGKKSVFDEELTNTSKKALK

SEQ ID NO: 96 - protein, 31 aa, Homo sapiens
  ATP-dependent RNA helicase DDX39A;Spliceosome RNA helicase DDX39B
GGDGAEAPAKKDVKGSYVSIHSSGFRDFLLK

SEQ ID NO: 97 - protein, 31 aa, Homo sapiens
  ATP-dependent RNA helicase DDX42
KLPQQSHSAFGATSSSSGFGKSAPPQLPSFY

SEQ ID NO: 98 - protein, 31 aa, Homo sapiens
  ATP-dependent RNA helicase DDX50
EEYYDGNTSSNSRQRSGWSSGRSGRSGRSGG

SEQ ID NO: 99 - protein, 31 aa, Homo sapiens
  Protein DEK
EDEDDEEEEEEEKEKSLIVEGKREKKKVERL

SEQ ID NO: 100 - protein, 17 aa, Homo sapiens
  ATP-dependent RNA helicase DHX36
MSYDYHQNWGRDGGPRS

SEQ ID NO: 101 - protein, 31 aa, Homo sapiens
  Pre-mRNA-splicing factor ATP-dependent RNA helicase PRP16
TDLDCQVGGLICKSKSAASEQHVFKAPAPRP

SEQ ID NO: 102 - protein, 17 aa, Homo sapiens
  Probable ATP-dependent RNA helicase DHX40
MSRFPAVAGRAPRRQEE

SEQ ID NO: 103 - protein, 31 aa, Homo sapiens
  Death-inducer obliterator 1
AVGKQPAPRNLVPKKSSFANVAAATPAIKKP

SEQ ID NO: 104 - protein, 31 aa, Homo sapiens
  Death-inducer obliterator 1
SVPMASPAPGRLGAMSAAPSQPNSQIRQNIR

SEQ ID NO: 105 - protein, 31 aa, Homo sapiens
  Death-inducer obliterator 1
QDVPKPVLTSVMVPKSILAKPSSSPDPRYLS

SEQ ID NO: 106 - protein, 31 aa, Homo sapiens
  Probable dimethyladenosine transferase
IGRRRGRQEQRRELKSAGGLMFNTGIGQHIL

SEQ ID NO: 107 - protein, 31 aa, Homo sapiens
  DNA methyltransferase 1-associated protein 1
PAVPETAGIKFPDFKSAGVTLRSQRMKLPSS

SEQ ID NO: 108 - protein, 31 aa, Homo sapiens
  DNA (cytosine-5)-methyltransferase 1
PPKPLSKPRTPRRSKSDGEAKPEPSPSPRIT

SEQ ID NO: 109 - protein, 31 aa, Homo sapiens
  Deoxynucleotidyltransferase terminal-interacting protein 2
KASIQAASAESSGQKSFAANGIQAHPESSTG

SEQ ID NO: 110 - protein, 31 aa, Homo sapiens
  Protein ECT2
TMYLYEKANTPELKKSVSMLSLNTPNSNRKR

SEQ ID NO: 111 - protein, 31 aa, Homo sapiens
  Histone-lysine N-methyltransferase EHMT1
GADVKVHRARKTMPKSVVGLHAASKDPREVR

SEQ ID NO: 112 - protein, 25 aa, Homo sapiens
  Alpha-endosulfine
TGDHIPTPQDLPQRKSSLVTSKLAG

SEQ ID NO: 113 - protein, 31 aa, Homo sapiens
  N-acetyltransferase ESCO2
EINRLPSANQGSPFKSALSTVSFYNQNKWYL

SEQ ID NO: 114 - protein, 31 aa, Homo sapiens
  ETS translocation variant 3
FNKLVMPNYPFINIRSSGVVPQSAPPVPTAS

SEQ ID NO: 115 - protein, 31 aa, Homo sapiens
  Protein FAM133B
ENWKKELEKHREKLLSGSESSSKKRQRKKKE

SEQ ID NO: 116 - protein, 31 aa, Homo sapiens
  Protein FAM178A
MKSLKKKHRSPERRKSLFIHENNEKNDRDRG

SEQ ID NO: 117 - protein, 31 aa, Homo sapiens
  Protein FAM64A
SGSPTHSLSQKSTRLSGAAPAHSAADPWEKE

SEQ ID NO: 118 - protein, 31 aa, Homo sapiens
  Protein FAM64A
EPGQQGLQAAARSAKSALGAVSQRIQESCQS

SEQ ID NO: 119 - protein, 31 aa, Homo sapiens
  Protein FAM76B
LSYKRVLQKTKEQRKSLGSSHSNSSSSSLTE

SEQ ID NO: 120 - protein, 31 aa, Homo sapiens
  Fanconi anemia group I protein
PLCYSFISYVQNKSKSLNYTGEKKEKPAAVA

SEQ ID NO: 121 - protein, 31 aa, Homo sapiens
  F-box/LRR-repeat protein 6
RSAEDWWWDRLAPRGSGYHLLQSDSMLLVLS

SEQ ID NO: 122 - protein, 31 aa, Homo sapiens
  Forkhead box protein K1
GSPIPHDPEFGSKLASVPEYRYSQSAPGSPV

SEQ ID NO: 123 - protein, 31 aa, Homo sapiens
  GAS2-like protein 3
DGAPQAKPVPAQKLKSALNLNQPVSVSSVSP

SEQ ID NO: 124 - protein, 24 aa, Homo sapiens
  Transcriptional repressor p66-alpha
VDRQREYLLDMIPPRSIPQSATWK

SEQ ID NO: 125 - protein, 31 aa, Homo sapiens
  G patch domain-containing protein 11
LLQKMGYKSGQALGKSGGGIVEPIPLNIKTG

SEQ ID NO: 126 - protein, 31 aa, Homo sapiens
  G patch domain-containing protein 11
GGIVEPIPLNIKTGKSGIGHEASLKRKAEEK

SEQ ID NO: 127 - protein, 31 aa, Homo sapiens
  G2 and S phase-expressed protein 1
GTKLLLPRAASVRGRSIPGAAEKPKKEIPAS

SEQ ID NO: 128 - protein, 31 aa, Homo sapiens
  Lymphoid-specific helicase
IELSPTGRPKRRTRKSINYSKIDDFPNELEK

SEQ ID NO: 129 - protein, 31 aa, Homo sapiens
  Embryonic stem cell-specific 5-hydroxymethylcytosine-binding protein
RQPYFIYFPQIKTEKSGSIGAADSPENWEKV

SEQ ID NO: 130 - protein, 23 aa, Homo sapiens
  High mobility group protein HMG-I/HMG-Y
MSESSSKSSQPLASKQEKDGTEK

SEQ ID NO: 131 - protein, 22 aa, Homo sapiens
  Non-histone chromosomal protein HMG-1
MPKRKVSSAEGAAKEEPKRRSA

SEQ ID NO: 132 - protein, 31 aa, Homo sapiens
  Non-histone chromosomal protein HMG-14
EGAAKEEPKRRSARLSAKPPAKVEAKPKKAA

SEQ ID NO: 133 - protein, 31 aa, Homo sapiens
  Non-histone chromosomal protein HMG-17
KAKVKDEPQRRSARLSAKPAPPKPEPKPKKA

SEQ ID NO: 134 - protein, 31 aa, Homo sapiens
  High mobility group nucleosome-binding domain-containing protein 3
SKVTKQEPTRRSARLSAKPAPPKPEPKPRKT

SEQ ID NO: 135 - protein, 31 aa, Homo sapiens
  High mobility group nucleosome-binding domain-containing protein 4
KAKVKDEPQRRSARLSAKPAPPKPEPRPKKA

SEQ ID NO: 136 - protein, 31 aa, Homo sapiens
  High mobility group nucleosome-binding domain-containing protein 5
QGDMRQEPKRRSARLSAMLVPVTPEVKPKRT

SEQ ID NO: 137 - protein, 31 aa, Homo sapiens
  Heterogeneous nuclear ribonucleoprotein A1; Heterogeneous nuclear ribonucleoprotein A1, N-terminally processed; Heterogeneous nuclear ribonucleoprotein A1-like 2
SSNFGPMKGGNFGGRSSGPYGGGGQYFAKPR

SEQ ID NO: 138 - protein, 31 aa, Homo sapiens
  Heterogeneous nuclear ribonucleoprotein A3
YSGQQQSNYGPMKGGSFGGRSSGSPYGGGYG

SEQ ID NO: 139 - protein, 31 aa, Homo sapiens
  Heterogeneous nuclear ribonucleoproteins C1/C2
DLDYDFQRDYYDRMYSYPARVPPPPPIARAV

SEQ ID NO: 140 - protein, 31 aa, Homo sapiens
  Heterogeneous nuclear ribonucleoprotein L-like
TPRGGGDGGGGGRSFSQPEAGGSHHKVSVSP

SEQ ID NO: 141 - protein, 31 aa, Homo sapiens
  Heterogeneous nuclear ribonucleoprotein U
QPQQQRGAAKEAAGKSSGPTSLFAVTVAPPG

SEQ ID NO: 142 - protein, 31 aa, Homo sapiens
  Homeobox protein Hox-B4
MKWKKDHKLPNTKIRSGGAAGSAGGPPGRPN

SEQ ID NO: 143 - protein, 31 aa, Homo sapiens
  Heterochromatin protein 1-binding protein 3
MDAILTEAIKACFQKSGASVVAIRKYIIHKY

SEQ ID NO: 144 - protein, 31 aa, Homo sapiens
  Jerky protein homolog
EELEAECFPVKPHNKSFAHILELVKEGSSCP

SEQ ID NO: 145 - protein, 31 aa, Homo sapiens
  Histone acetyltransferase KAT6A
QGQMPVKGHISIRSKSAPLPSAAAHQQQLYG

SEQ ID NO: 146 - protein, 31 aa, Homo sapiens
  Lysine-specific demethylase 2B
PRPPLGSSLSPWWRSSLTYFQQQLKPGKEDK

SEQ ID NO: 147 - protein, 31 aa, Homo sapiens
  Lysine-specific demethylase 2B
SPRPPLGSSLSPWWRSSLTYFQQQLKPGKED

SEQ ID NO: 148 - protein, 31 aa, Homo sapiens
  KH domain-containing, RNA-binding, signal transduction-associated protein 1
RRDDPAARMSRSSGRSGSMDPSGAHPSVRQT

SEQ ID NO: 149 - protein, 31 aa, Homo sapiens
  Kinesin-like protein KIFC1
GLKNQKPVPAVPVQKSGTSGVPPMAGGKKPS

SEQ ID NO: 150 - protein, 31 aa, Homo sapiens
  Lysine-rich nucleolar protein 1
YFADVSPLRATSPSKSVAHGQAPEMPLVKKK

SEQ ID NO: 151 - protein, 31 aa, Homo sapiens
  LIM/homeobox protein Lhx9
GEYPPQLSYTELAAKSGGLALPYFNGTGTVQ

SEQ ID NO: 152 - protein, 19 aa, Homo sapiens
  DNA ligase;DNA ligase 1
MQRSIMSFFHPKKEGKAKK

SEQ ID NO: 153 - protein, 31 aa, Homo sapiens
  DNA ligase 3
VKGASFVTSTNPRKFSGFSAKPNNSGEAPSS

SEQ ID NO: 154 - protein, 31 aa, Homo sapiens
  DNA ligase 3
KLTTTGQVTSPVKGASFVTSTNPRKFSGFSA

SEQ ID NO: 155 - protein, 31 aa, Homo sapiens
  Protein LLP homolog
EKRKKNAPKEASRLKSILKLDGDVLMKDVQE

SEQ ID NO: 156 - protein, 31 aa, Homo sapiens
  Prelamin-A/C; Lamin-A/C
SGSSASSVTVTRSYRSVGGSGGGSFGDNLVT

SEQ ID NO: 157 - protein, 27 aa, Homo sapiens
  Prelamin-A/C; Lamin-A/C
METPSQRRATRSGAQASSTPLSPTRIT

SEQ ID NO: 158 - protein, 31 aa, Homo sapiens
  Microtubule-associated protein; Microtubule-associated protein 4
KTEGKPAEVKKMTAKSVPADLSRPKSTSTSS

SEQ ID NO: 159 - protein, 31 aa, Homo sapiens
  MAP7 domain-containing protein 1
LPKHVDSIINKRLSKSSATLWNSPSRNRSLQ

SEQ ID NO: 160 - protein, 31 aa, Homo sapiens
  Microtubule-associated protein RP/EB family member 1
SLVAPALNKPKKPLTSSSAAPQRPISTQRTA

SEQ ID NO: 161 - protein, 31 aa, Homo sapiens
  Methyl-CpG-binding domain protein 2
GGGAPRREPVPFPSGSAGPGPRGPRATESGK

SEQ ID NO: 162 - protein, 31 aa, Homo sapiens
  Methyl-CpG-binding domain protein 4
LKGIPIKKTKKGCRKSCSGFVQSDSKRESVC

SEQ ID NO: 163 - protein, 31 aa, Homo sapiens
  Methyl-CpG-binding domain protein 4
MPPSSSSELQESRGLSNFTSTHLLLKEDEGV

SEQ ID NO: 164 - protein, 31 aa, Homo sapiens
  Protein MCM10 homolog
YKKLSAKRADLQSTFSGGRIPKKFARRGTSL

SEQ ID NO: 165 - protein, 31 aa, Homo sapiens
  MAX gene-associated protein
NRQATFSGRTKSSYKSILPYPVSPKQKYSHV

SEQ ID NO: 166 - protein, 31 aa, Homo sapiens
  Antigen KI-67
DVKSQKENVLQYCRKSGLQTDYATEKESADG

SEQ ID NO: 167 - protein, 31 aa, Homo sapiens
  Antigen KI-67
PNTPLKRGEAPTKRKSLVMHTPPVLKKIIKE

SEQ ID NO: 168 - protein, 31 aa, Homo sapiens
  Antigen KI-67
EISSVKLVSRYGELKSVPTTQCLDNSKKNES

SEQ ID NO: 169 - protein, 31 aa, Homo sapiens
  Antigen KI-67
RSQHDILQMICSKRRSGASEANLIVAKSWAD

SEQ ID NO: 170 - protein, 31 aa, Homo sapiens
  Protein AF-9
SAKKRKKSSSEALFKSFSSAPPLILTCSADK

SEQ ID NO: 171 - protein, 31 aa, Homo sapiens
  Protein AF-9
KEHKEKPSKDSREHKSAFKEPSRDHNKSSKE

SEQ ID NO: 172 - protein, 20 aa, Homo sapiens
  DNA-3-methyladenine glycosylase
MPARSGAQFCRRMGQKKQRP

SEQ ID NO: 173 - protein, 31 aa, Homo sapiens
  DNA-3-methyladenine glycosylase
RERCLGPPTTPGPYRSIYFSSPKGHLTRLGL

SEQ ID NO: 174 - protein, 31 aa, Homo sapiens
  DNA mismatch repair protein Msh6
ATSISSETKNTLRAFSAPQNSESQAHVSGGG

SEQ ID NO: 175 - protein, 31 aa, Homo sapiens
  DNA mismatch repair protein Msh6
EEYIPLDSDTVSTTRSGAIFTKAYQRMVLDA

SEQ ID NO: 176 - protein, 31 aa, Homo sapiens
  Metastasis-associated protein MTA1
YLETHPRPPKPDPVKSVSSVLSSLTPAKVAP

SEQ ID NO: 177 - protein, 31 aa, Homo sapiens
  Metal-response element-binding transcription factor 2
HYGLSDSRKRTRTGRSWPAAIPHLRRRRGRL

SEQ ID NO: 178 - protein, 31 aa, Homo sapiens
  Metal-response element-binding transcription factor 2
SREVSNGIEKKGKKKSVGRPPGPYTRKMIQK

SEQ ID NO: 179 - protein, 31 aa, Homo sapiens
  Nuclear receptor coactivator 7
PPMFLCIKVGKPMRKSFATHTAAMVQQYGKR

SEQ ID NO: 180 - protein, 31 aa, Homo sapiens
  Nuclear receptor corepressor 2
PVSPPEGMTEPGHSRSAVYPLLYRDGEQTEP

SEQ ID NO: 181 - protein, 31 aa, Homo sapiens
  Negative elongation factor E
NIARKQPMLDAATGKSVWGSLAVQNSPKGCH

SEQ ID NO: 182 - protein, 31 aa, Homo sapiens
  Negative elongation factor E
MDTATATEQAKQLVKSGAISAIKAETKNSGF

SEQ ID NO: 183 - protein, 31 aa, Homo sapiens
  Nuclear factor 1; Nuclear factor 1 A-type
EPGMPSPTTLKKSEKSGFSSPSPSQTSSLGT

SEQ ID NO: 184 - protein, 31 aa, Homo sapiens
  Nuclear factor 1; Nuclear factor 1 A-type
ESSSYYSMSPGAMRRSLPSTSSTSSTKRLKS

SEQ ID NO: 185 - protein, 31 aa, Homo sapiens
  Nuclear factor 1; Nuclear factor 1 A-type
PTYSTPSTSPANRFVSVGPRDPSFVNIPQQT

SEQ ID NO: 186 - protein, 31 aa, Homo sapiens
  Nuclear factor related to kappa-B-binding protein
ITVPLSVISQPMKGKSVVTAPIIKGNLGANL

SEQ ID NO: 187 - protein, 31 aa, Homo sapiens
  NF-kappa-B inhibitor-interacting Ras-like protein 2
PFVYLASKMTQPQSKSAFPLSRKNKGSGSLD

SEQ ID NO: 188 - protein, 31 aa, Homo sapiens
  Nucleolar and coiled-body phosphoprotein 1
PYSSVPPPSAPPPKKSLGTQPPKKAVEKQQP

SEQ ID NO: 189 - protein, 31 aa, Homo sapiens
  Nucleolar and coiled-body phosphoprotein 1
MVATTKPKATAKAALSLPAKQAPQGSRDSSS

SEQ ID NO: 190 - protein, 31 aa, Homo sapiens
  Probable 28S rRNA (cytosine(4447)-C(5))-methyltransferase
SPEAKPLPGKLPKGISAGAVQTAGKKGPQSL

SEQ ID NO: 191 - protein, 31 aa, Homo sapiens
  Nucleolar protein 9
RRFPAGGKRGRGAKGSGRPLPGRKRQPWPPP

SEQ ID NO: 192 - protein, 31 aa, Homo sapiens
  Histone-lysine N-methyltransferase, H3 lysine-36 and H4 lysine-20 specific
PLERPLGTADPRLDKSIGAASPRPQSLEKTS

SEQ ID NO: 193 - protein, 31 aa, Homo sapiens
  Nuclear fragile X mental retardation-interacting protein 1
WYWRQSSDRFPRHQKSFNPAVKNSYYPRKYD

SEQ ID NO: 194 - protein, 31 aa, Homo sapiens
  Nuclear mitotic apparatus protein 1
KKAAPASTKQADRRQSMAFSILNTPKKLGNS

SEQ ID NO: 195 - protein, 31 aa, Homo sapiens
  Nuclear mitotic apparatus protein 1
VEEPDSANSSFYSTRSAPASQASLRATSSTQ

SEQ ID NO: 196 - protein, 31 aa, Homo sapiens
  Nucleolar and spindle-associated protein 1
NKGGVRTPVPPRGRLSVASTPISQRRSQGRS

SEQ ID NO: 197 - protein, 31 aa, Homo sapiens
  Nucleolar and spindle-associated protein 1
SVASTPISQRRSQGRSCGPASQSTLGLKGSL

SEQ ID NO: 198 - protein, 31 aa, Homo sapiens
  Nucleolar and spindle-associated protein 1
SSGNRDSKVPSEGKKSLYTDESSKPGKNKRT

SEQ ID NO: 199 - protein, 31 aa, Homo sapiens
  Nucleolar and spindle-associated protein 1
PASQSTLGLKGSLKRSAISAAKTGVRFSAAT

SEQ ID NO: 200 - protein, 31 aa, Homo sapiens
  Origin recognition complex subunit 1
IREERTLTPISGGQRSSVVPSVILKPENIKK

SEQ ID NO: 201 - protein, 31 aa, Homo sapiens
  Polyadenylate-binding protein 2
AAAAAAAAGAAGGRGSGPGRRRHLVPGAGGE

SEQ ID NO: 202 - protein, 31 aa, Homo sapiens
  Poly [ADP-ribose] polymerase 1
EVKAEPVEVVAPRGKSGAALSKKSKGQVKEE

SEQ ID NO: 203 - protein, 31 aa, Homo sapiens
  Protein polybromo-1
NLAAARLTGPSHSKGSLGEERNPTSKYYRNK

SEQ ID NO: 204 - protein, 31 aa, Homo sapiens
  Protein-L-isoaspartate O-methyltransferase; Protein-L-isoaspartate(D-aspartate) O-methyltransferase
VVLYLLRVCLAMAWKSGGASHSELIHNLRKN

SEQ ID NO: 205 - protein, 31 aa, Homo sapiens
  Retrotransposon-derived protein PEG10
PNNNNNNNSKHTGHKSACVPNMTERRRDELS

SEQ ID NO: 206 - protein, 28 aa, Homo sapiens
  Pescadillo homolog
MGGLEKKKYERGSATNYITRNKARKKLQ

SEQ ID NO: 207 - protein, 31 aa, Homo sapiens
  Polyhomeotic-like protein 2
GFVIQEGAEPFPVGRSSLLVGNLKKKYAQGF

SEQ ID NO: 208 - protein, 31 aa, Homo sapiens
  Polyhomeotic-like protein 2
KAGAATHNRRRASKASLPPLTKDTKKQPTGT

SEQ ID NO: 209 - protein, 27 aa, Homo sapiens
  PHD Finger Protein 10
ATPRKDGPKRSVLSKSVPGYKVEEKSP

SEQ ID NO: 210 - protein, 31 aa, Homo sapiens
  Lysine-specific demethylase PHF2
ALTKMEPPKKGKATKSVLSVPNKDVVHMQND

SEQ ID NO: 211 - protein, 31 aa, Homo sapiens
  PIN2/TERF1-interacting telomerase inhibitor 1
HGQETTDSSDKKEKKSFSLEEKSKISKNRVH

SEQ ID NO: 212 - protein, 31 aa, Homo sapiens
  Pituitary homeobox 1
DVYAAGYSYNNWAAKSLAPAPLSTKSFTFFN

SEQ ID NO: 213 - protein, 31 aa, Homo sapiens
  Proline-rich nuclear receptor coactivator 1
PFKNTENIKNSHLKKSAFLTEVSQKENYAGA

SEQ ID NO: 214 - protein, 31 aa, Homo sapiens
  Proline-rich nuclear receptor coactivator 1
CLTPQPRAPAALPNRSLAVAGGTPRAAPKKR

SEQ ID NO: 215 - protein, 31 aa, Homo sapiens
  DNA polymerase; DNA polymerase alpha catalytic subunit
PQITPPPVMILKKKRSIGASPNPFSVHTATA

SEQ ID NO: 216 - protein, 31 aa, Homo sapiens
  Polymerase delta-interacting protein 3
PAEVDPDTILKALFKSSGASVTTQPTEFKIK

SEQ ID NO: 217 - protein, 31 aa, Homo sapiens
  Ribonucleases P/MRP protein subunit POP1
RAAEISAMLKAVTQKSSNSLVFQTLPRHMRR

SEQ ID NO: 218 - protein, 31 aa, Homo sapiens
  Ribonucleases P/MRP protein subunit POP1
TLSSGFVADRGVKHHSGGEKPFQAQKQEPHP

SEQ ID NO: 219 - protein, 18 aa, Homo sapiens
  Ribonuclease P protein subunit p29
MKSVIYHALSQKEANDSD

SEQ ID NO: 220 - protein, 31 aa, Homo sapiens
  Periphilin-1
RQPEYRDMRDGFRRKSFYSSHYARERSPYKR

SEQ ID NO: 221 - protein, 31 aa, Homo sapiens
  Peptidyl-prolyl cis-trans isomerase-like 2
ERKTQLKVAPETKVKSSQPQAGSQGPQTFRQ

SEQ ID NO: 222 - protein, 31 aa, Homo sapiens
  Protein phosphatase 1D
SGPLMKKHRRNGLSRSSGAQPASLPTTSQRK

SEQ ID NO: 223 - protein, 31 aa, Homo sapiens
  Proline-rich protein PRCC
TTTTPSPSAIKAAAKSAALQVTKQITQEEDD

SEQ ID NO: 224 - protein, 31 aa, Homo sapiens
  DNA-dependent protein kinase catalytic subunit
FAHKRSERLQRAPLKSVGPDFGKKRLGLPGD

SEQ ID NO: 225 - protein, 31 aa, Homo sapiens
  Protein PRRC2A
KKYSSLNLFDTYKGKSLEIQKPAVAPRHGLQ

SEQ ID NO: 226 - protein, 31 aa, Homo sapiens
  Polymerase I and transcript release factor
ERREKLKTSRDKLRKSFTPDHVVYARSKTAV

SEQ ID NO: 227 - protein, 31 aa, Homo sapiens
  Rac GTPase-activating protein 1
RQFVDGPPGPVKKTRSIGSAVDQGNESIVAK

SEQ ID NO: 228 - protein, 19 aa, Homo sapiens
  DNA repair and recombination protein RAD54B
MRRSAAPSQLQGNSFKKPK

SEQ ID NO: 229 - protein, 31 aa, Homo sapiens
  Retinoic acid-induced protein 1
GSKLSDRPLHALKRKSAFMAPVPTKKRNLVL

SEQ ID NO: 230 - protein, 31 aa, Homo sapiens
  RNA-binding protein 27
QSAPSTVHGGIQKMMSKPQTSGAYVLNKVPV

SEQ ID NO: 231 - protein, 31 aa, Homo sapiens
  RNA-binding protein 33
PAGPHAHSPVPPGIKSIQGIHPAKKAIMHGR

SEQ ID NO: 232 - protein, 31 aa, Homo sapiens
  RNA-binding protein 34
QGLNFTSKTAEGHPKSLFIGEKAVLLKTKKK

SEQ ID NO: 233 - protein, 31 aa, Homo sapiens
  RNA-binding motif protein, X chromosome; RNA-binding motif protein, X chromosome, N-terminally processed
GGSYRDSYESYGNSRSAPPTRGPPPSYGGSS

SEQ ID NO: 234 - protein, 31 aa, Homo sapiens
  DNA-binding protein RFX5
KKSGGSGERNSTPLKSAAAMESAQSSRLPWE

SEQ ID NO: 235 - protein, 26 aa, Homo sapiens
  E3 ubiquitin-protein ligase RNF168
VSKSAHSLQPSISQKSVFQMFQRCTK

SEQ ID NO: 236 - protein, 30 aa, Homo sapiens
  60S ribosomal protein L31
MAPAKKGGEKKKGRSAINEVVTREYTINIH

SEQ ID NO: 237 - protein, 31 aa, Homo sapiens
  60S ribosomal protein L8
CLEEKPGDRGKLARASGNYATVISHNPETKK

SEQ ID NO: 238 - protein, 31 aa, Homo sapiens
  Active regulator of SIRT1
QAQKLRNSAKGKVPKSALDEYRKRECRDHLR

SEQ ID NO: 239 - protein, 31 aa, Homo sapiens
  Ribosomal protein S6 kinase; Ribosomal protein S6 kinase alpha-4
FMAFNRGKREGFFLKSVENAPLAKRRKQKLR

SEQ ID NO: 240 - protein, 31 aa, Homo sapiens
  Ribosomal RNA processing protein 1 homolog B
GLNRNMTAEFKKTDKSILVSPTGPSRVAFDP

SEQ ID NO: 241 - protein, 31 aa, Homo sapiens
  Ribosomal RNA processing protein 1 homolog B
DTPFLPKPLFFRRAKSSTATHPPGPAVQLNK

SEQ ID NO: 242 - protein, 31 aa, Homo sapiens
  RNA polymerase-associated protein RTF1 homolog
EERAEALDRQRTKNISAISYINQRNREWNIV

SEQ ID NO: 243 - protein, 29 aa, Homo sapiens
  RNA polymerase-associated protein RTF1 homolog
ITSKAPPAKDGAPRRSLNLEDYKKRRGLI

SEQ ID NO: 244 - protein, 31 aa, Homo sapiens
  U4/U6.U5 tri-snRNP-associated protein 1
ETTVQKVARVKAPNKSLPSAVYCIEDKMAID

SEQ ID NO: 245 - protein, 31 aa, Homo sapiens
  Protein SCAF11
YKDQNENRWQNRKPLSGNSNSSGSESFKFVE

SEQ ID NO: 246 - protein, 31 aa, Homo sapiens
  Plasminogen activator inhibitor 1 RNA-binding protein
KKEAGGGGVGGPGAKSAAQAAAQTNSNAAGK

SEQ ID NO: 247 - protein, 31 aa, Homo sapiens
  Plasminogen activator inhibitor 1 RNA-binding protein
SRGKREFDRHSGSDRSSFSHYSGLKHEDKRG

SEQ ID NO: 248 - protein, 31 aa, Homo sapiens
  Survival of motor neuron-related-splicing factor 30
NNRAYSKNKKGQVKRSIFASPESVTGKVGVG

SEQ ID NO: 249 - protein, 31 aa, Homo sapiens
  Spindlin-1
SANMMKKRTSHKKHRSSVGPSKPVSQPRRNI

SEQ ID NO: 250 - protein, 31 aa, Homo sapiens
  Protein SPT2 homolog
SGPGRSISGSIPAGRTVSNSVPGRPVSSLGP

SEQ ID NO: 251 - protein, 31 aa, Homo sapiens
  Protein SPT2 homolog
QEPPKVESKPKVPLKSAPPPMNFTDLLRLAE

SEQ ID NO: 252 - protein, 31 aa, Homo sapiens
  Protein SPT2 homolog
ASRTQKSAVEHKAKKSLSHPSHSRPGPMVTP

SEQ ID NO: 253 - protein, 31 aa, Homo sapiens
  Helicase SRCAP
RLVGTTNQGDQRILRSSAPPSLAGPAVSHRG

SEQ ID NO: 254 - protein, 26 aa, Homo sapiens
  Protein SREK1IP1
HHKKEKKKRKKEKHSSTPNSSEFSRK

SEQ ID NO: 255 - protein, 17 aa, Homo sapiens
  Serine/arginine-rich splicing factor 1
MSGGGVIRGPAGNNDCR

SEQ ID NO: 256 - protein, 31 aa, Homo sapiens
  SUN domain-containing protein 1
NRAARTTKQRRSTNKSAFSINHVSRQVTSSG

SEQ ID NO: 257 - protein, 31 aa, Homo sapiens
  Transcription factor 19
RPQPLTFSPSWGGPKSLPVPAPPGEVGTTPS

SEQ ID NO: 258 - protein, 31 aa, Homo sapiens
  Transcription factor 7-like 2
RKRDKQPGETNGEKKSAFATYKVKAAASAHP

SEQ ID NO: 259 - protein, 31 aa, Homo sapiens
  Treacle protein
RDKASGDVKEKKGKGSLGSQGAKDEPEEELQ

SEQ ID NO: 260 - protein, 31 aa, Homo sapiens
  Treacle protein
SDGEVPTAVAPAQEKSLGNILQAKPTSSPAK

SEQ ID NO: 261 - protein, 31 aa, Homo sapiens
  Treacle protein
GKGLQVKAASVPVKGSLGQGTAPVLPGKTGP

SEQ ID NO: 262 - protein, 31 aa, Homo sapiens
  Treslin
RSAKKRRKNALIRHKSIAEVSQNLRQIEIPK

SEQ ID NO: 263 - protein, 31 aa, Homo sapiens
  Treslin
DNFKKNKGYHKLLTKSVAETPVHKQISKRLL

SEQ ID NO: 264 - protein, 31 aa, Homo sapiens
  Lamina-associated polypeptide 2, isoform alpha; Thymopoietin; Thymopentin
GYYKDIVENICGREKSGIQPLCPERSHISDQ

SEQ ID NO: 265 - protein, 31 aa, Homo sapiens
  TOX high mobility group box family member 4
VRINLQQQPPPLQIKSVPLPTLKMQTTLVPP

SEQ ID NO: 266 - protein, 31 aa, Homo sapiens
  Targeting protein for Xklp2
FKKLALAGIGQPVKKSVSQVTKSVDFHFRTD

SEQ ID NO: 267 - protein, 31 aa, Homo sapiens
  E3 ubiquitin-protein ligase TRIP12
AARFSPKVSLPKTKLSLPGSSKSETSKPGPS

SEQ ID NO: 268 - protein, 31 aa, Homo sapiens
  E3 ubiquitin-protein ligase TRIP12
VDNQAKSPTTTQSPKSSFLASLNPKTWGRLS

SEQ ID NO: 269 - protein, 31 aa, Homo sapiens
  Zinc finger transcription factor Trps1
ETKGFLQGAPAGGEKSGALPQQYPASGENKS

SEQ ID NO: 270 - protein, 31 aa, Homo sapiens
  Zinc finger transcription factor Trps1
PSSEVAKPSEKNSNKSIPALQSSDSGDLGKW

SEQ ID NO: 271 - protein, 31 aa, Homo sapiens
  Teashirt homolog 2
QDALSKSLQQNLPSRSVSKPSLFSSVQLYRQ

SEQ ID NO: 272 - protein, 31 aa, Homo sapiens
  Ubiquitin carboxyl-terminal hydrolase 1
RPSQKKSRVKINWLKSATKQPSILSKFCSLG

SEQ ID NO: 273 - protein, 31 aa, Homo sapiens
  WW domain-binding protein 11
SEDDSAVPLAKAAPKSGPSVPVSVQTKDDVY

SEQ ID NO: 274 - protein, 31 aa, Homo sapiens
  WD repeat and HMG-box DNA-binding protein 1
NSFSKSTNSSDVSAKSGAVTFSSQGRVNPFK

SEQ ID NO: 275 - protein, 29 aa, Homo sapiens
  Histone-lysine N-methyltransferase NSD2
NRASTAASSALGFSKSSSPSASLTENEVK

SEQ ID NO: 276 - protein, 31 aa, Homo sapiens
  Histone-lysine N-methyltransferase NSD3
PPPVKIAWKTAAARKSLPASITMHKGSLDLQ

SEQ ID NO: 277 - protein, 27 aa, Homo sapiens
  Protein Wiz
MDLGSPSLPKKSLPVPGALEQVASRLS

SEQ ID NO: 278 - protein, 31 aa, Homo sapiens
  DNA repair protein complementing XP-C cells
EPVLGDVRESTAFSRSLLPVKPVEIEIETPE

SEQ ID NO: 279 - protein, 31 aa, Homo sapiens
  YLP motif-containing protein 1
SALPYSSFSSDQGLGESSAAPSQPITAVKDM

SEQ ID NO: 280 - protein, 31 aa, Homo sapiens
  Zinc finger and BTB domain-containing protein 5
SGYQGGEQFGMDFSRSGLGLHSSFSRVMIGS

SEQ ID NO: 281 - protein, 17 aa, Homo sapiens
  Zinc finger CCHC-type and RNA-binding motif-containing protein 1
MSGGLAPSKSTVYVSNL

SEQ ID NO: 282 - protein, 31 aa, Homo sapiens
  Zinc finger protein 37 homolog
NCVKRKSDAAKEHKKSFNHSLSDTRKGKKQT

SEQ ID NO: 283 - protein, 31 aa, Homo sapiens
  Zinc finger protein 62 homolog
THSGEKNCKCDECGKSFNYSSVLDQHKRIHT

SEQ ID NO: 284 - protein, 31 aa, Homo sapiens
  Zinc finger protein 62 homolog
IHPGKKAHECKECGKSFSYNSLLLQHRTIHT

SEQ ID NO: 285 - protein, 31 aa, Homo sapiens
  Zinc finger MYM-type protein 4
HRDGFPQPRRRGRKKSIVAVEPRSLIQGAFQ

SEQ ID NO: 286 - protein, 31 aa, Homo sapiens
  Zinc finger protein 217
NTAAEFGEPLPKRLKSSVVALDVDQPGANYR

SEQ ID NO: 287 - protein, 31 aa, Homo sapiens
  Zinc finger protein 22
IHTGKKSHKCADCGKSFFQSSNLIQHRRIHT

SEQ ID NO: 288 - protein, 31 aa, Homo sapiens
  Zinc finger protein 281
SQGNTSSSRRKTKSKSIAIENKEQKTGKTNE

SEQ ID NO: 289 - protein, 31 aa, Homo sapiens
  Zinc finger protein 282
PYSCPECGKSFGVRKSLIIHHRSHTKERPYE

SEQ ID NO: 290 - protein, 31 aa, Homo sapiens
  Zinc finger protein 286A;Putative zinc finger protein 286B
TDHKHDVYWKSFNQKSVLITEDRVPKGSYAF

SEQ ID NO: 291 - protein, 31 aa, Homo sapiens
  Zinc finger protein 302;Zinc finger protein 181
LLNSNKSGAAFNQSKSLTLPQTCNREKIYTC

SEQ ID NO: 292 - protein, 31 aa, Homo sapiens
  Zinc finger protein 316
YHAGERPHRCADCGKSFVYGSHLARHRRTHT

SEQ ID NO: 293 - protein, 31 aa, Homo sapiens
  Zinc finger protein 432
SCEINNSTKFSGDGKSFLHGNYEELYSAAKF

SEQ ID NO: 294 - protein, 31 aa, Homo sapiens
  Zinc finger protein 763; Zinc finger protein 439; Zinc finger protein 440
IHTGEKPCECKQCGKSFSYSATHRIHKRTHT

SEQ ID NO: 295 - protein, 31 aa, Homo sapiens
  Zinc finger protein 462
RQQQEGTNLPDVPNKSAPSPTSNSTYLTMNA

SEQ ID NO: 296 - protein, 31 aa, Homo sapiens
  Zinc finger protein 512B
VTKAMPVTKPITVTKSVPVTKPVPVTKPITV

SEQ ID NO: 297 - protein, 31 aa, Homo sapiens
  Zinc finger protein 562
VHTGKKSEKTKNCGKSFTNFSQLSAHAKTHK

SEQ ID NO: 298 - protein, 31 aa, Homo sapiens
  Zinc finger protein 614
KICIPNEYRKGSTVKSSLITHQQTHTEEKSY

SEQ ID NO: 299 - protein, 31 aa, Homo sapiens
  Zinc finger protein 615
SSGLKNSAEFNRDGKSLFHANHKQFYTEMKF

SEQ ID NO: 300 - protein, 31 aa, Homo sapiens
  Zinc finger protein 622
YKTDWHRYNLRRKVASMAPVTAEGFQERVRA

SEQ ID NO: 301 - protein, 31 aa, Homo sapiens
  Zinc finger protein 644
KKTFMKDSVVGSSKKSATYICKMCPFTTSAK

SEQ ID NO: 302 - protein, 31 aa, Homo sapiens
  Zinc finger protein 721
VHTREKPYKCEDRGRSFGWSTNLNEYKKIHT

SEQ ID NO: 303 - protein, 31 aa, Homo sapiens
  Zinc finger protein 766
KPNRCHECGKTVRDKSGLAEHWRIRTGEKPY

SEQ ID NO: 304 - protein, 31 aa, Homo sapiens
  Zinc finger protein 768
RPFSCGICGKSFSQRSALIPHARSHAREKPF

SEQ ID NO: 305 - protein, 31 aa, Homo sapiens
  Zinc finger protein 92;Zinc finger protein 429
RHTGKKPFKCKNRGKSFCMLSQLTQHKKIHT

SEQ ID NO: 306 - protein, 20 aa, Homo sapiens
  Zinc finger and SCAN domain-containing protein 29
MMAKSALRENGTNSETFRQR

SEQ ID NO: 307 - protein, 31 aa, Homo sapiens
  Zinc finger and SCAN domain-containing protein 29
QEQMNPKEKLKPFQRSGLPFPKSGVVSRLEQ

SEQ ID NO: 308 - protein, 31 aa, Homo sapiens
  ZZ-type zinc finger-containing protein 3
NGLDESFCGRTLRNRSIAHPEEISSNSQVRS

SEQ ID NO: 309 - protein, 31 aa, Homo sapiens
  ATP-dependent RNA helicase DDX39A; Spliceosome RNA helicase DDX39B
PQESTPAPPKKDIKGSYVSIHSSGFRDFLLK